European Patent Specification EP 3 492 595 B1, published December 20, 2023. Title: Resistenzgen gegen Rizomania. Applicant: KWS SAAT SE. The sequence listing filed with the application follows.

SEQUENCE LISTING (7 sequences)

SEQ ID NO: 1 - DNA, 5009 bp, Beta vulgaris
caaatcttctggcatcaatggcggtgttgccgttcatcaatttaacatcaatggaggtaagagtcatgttttttcaacaatataaaacttatacttcctctgttctgttttaaatgaaacgtttgttttctcacgcaacccaacccacttttttaataataaatatttttagttgtgtgcacgtaaaaaatataaaaaagttataatttgatagtatcttgtttgagattgtgattattaagagagtcaagtctcacaatattcgaaagtctacgtaatccacctcaaattgacgaagaaaacaagcaggaaaggattaagtaagttcgtggaaccactagaattgattttcaaatatagctctacctaatatatggcctacttttaattttaaataaggagaaggtaatgtgattagaaacaaattggtcttaaattattcattaagcttaataatgtataaacataatcaagtgctatcttcttttcagggccgtcttgaagattttggggcccggttctattatgaaaattgggcccctaaatttatagaaaataaagatggaaggttagagttctaaagatagaaagttgaaaatctaaatataaatcattgacaaatttattaagggtgagaaacaagggtgttttcttcaaatatgaagcaaaattttcaaaataatacttcctccgtttctaaataagtgcaacatttgcataatgtttactattcacagtttaaactttaattagctttggtgatttacattttaggaaaaaacatagtcatgtgggatcttgttagattcgtctgaatgtgaatttttttaatatcaactttttataatttttacttattgataattgaagatattaatggttaaaataatgcattggcaaacgtgaaaacaagaagtgttgcacttatttagaaacggaggaagtatattttgggcctttataattttggagaccctgcgctgttgggctccttgcacaccttcatctacccctctgcttcttttgatacaatttttcagcgacatgattgtcgattgatgcatatattattgtatactcgatccatattgtttaagatgaattgtttgtctttgatggtctccaatgcatattttgtatacttaggaattctaattatgtactattagtagacattgagatgaatacataattgccataatgaagtatgattattttagttatatactttctccattccaaatatataaatgtaacacttgtgtactttatgcgtactaatgcataacaacgtgcactctcatgtgtttaattatatactttttgagagaagtgttacattggggaccatgggactgtgtataatttgaccgcaaaatcgaagtgtcgcatttgattgaaaatggagagagtagtatatagatggaacacagcagagactgctggtcatctttggccaacaaacccaaaattgatattaatcccttattcaggtcatttcatctttttgacacaaaatggatgttgtaggcactgcgctatctgctgcccaatctctgtttgcagccctgcaaagttctgagctcaaagagatcctctcgatctttggctacaaatcccgacttgatgacctccaacgcactgtctctaccatcaacgctgtattccgtgatgctgagaccaaacaggagctcactcatgaagcacagcattggctcgaggaactcaaggatgctgtctttgaagcagatgatctgttcgacgagtttgtcactcttgccgagcagaagcaacttgtagaggctggtggcagtctttccaaaaagatgcgccaattcttttctgattccaacccccttggcattgcttataggatgtcacgaggggttaagaagatcaagaagaagttggatgctatcgcttacaatcatcaatttagctttaagattgatcttgagcctatgaaagagagaaggctagagactggttctgtcgtgaacgcaggtgatatcattggaagagaggacgacttggagaagattgtaggtttgttgcttgattctaacatccaacgtgatgtgtctttccttactattgtgggaatgggagggttgggtaaaactgctcttgcccaactcgtgtacaatgatccaagggtcagaactgcttttccattgagatgttggaattgtgtgtctgatcaagatcaaaagcaactagatgtgaaagaaattttgggtaagattctggctacagctactggtaagaatcatgagggttcaaccatggatcaggtgcaaacccaactacgagaacaactatgtggcaagagatacttgcttgttttggatgatgtatggaatgagaatcctaatcaattgcgtgatctggtagaattcttcatgggaggtcgaagcagaaattggattgtggtaactacgcgttcgcacgagacagcgagaattataagagatggtccattgcacaagctccaaggtttgtctgaggaaaactcttggcgtttatttgtcaggtggaccttcggatcagtgcaagcaaaattccctaatgactttatcatgattgcacgagatatagttgacaaatgtgctcgaaaccctctggctataagagtggtaggaagtcttttgtgtggtcaagacaagagtaagtggctttcatttcatgagatcgatttaggcaacattagaaagagccataatgatatcatgccaatactgaacctaagttaccatcatcttgaacctccaattaagagatgctttagttattgtgcagtgtttccaaaggatttccttatagggaagcagacgctgataaacctctggatggcacaaggttatattgttccgttagacaaagatcaaagcatagatgatgctagtgaggaatacatatcaattttgttgcggagatgttttttcgaaaatgtcggagcagaaaaagatggtgttattaagatccatgatctcatgcatgatattgctcaaaatgtcatggggaaggagctttgtacgactaaaaacattagtggcagcttggataaaagtgttcgccatctatctcttgccagaactagttttgcaagatactctttcaatgcaactcatattcgctcctatttctgtgctggctactggtgtcaggatgctgagataaaccagttttcagttgaggcattagtaccaaactgtttgtacctaagggcaatggacctcgcttggtcgaagataaaaagtttaccagactcgattggtggattgttgcatttgaggtacttagatctttcgtataacgaagatctggaagtacttccaaactcaattgctaaactatataatctacaaaccttacaattgaagggttgcaagagattggaagggttaccaaaacatttgagcaggctggttaagcttcaaactttggatatacatggttgcaacaatgtaacttatatgcccaaaggcatgggtaagttgacttgccttcacactctcagtaagtttatagtgggtggagaagggagttgttcaagttggaagcaatgttttgatgggttggaagatctaaaggctctcaataacctaaagggtcatctggaaatccaaatcaggtggcccaaaaatactacagatgctgtcaaagaagatgttacgagggaaggattatacctgaatcataaggaacatctcaatcacattgtggttgattttagatgtgaggagggtggtggaagaatggatgatgaggaagcaagaagattgatggaagagttgcggccacatccttatcttgaaaatttggctgtgaaagcatattatggtgtgaaaatgcctggttgggcaacccttctcccaaatcttacagagctttttctttctgattgtggggaactggagaaccttccatgcctgggaaacttggatcatctaaaagtcctccgactttcgcatttggcaaaattggagtacattgaagaagatagctcatcagctaatttcaggtgtaggcctggaccagaaagtgcaggactatcattatacttcccctcccttgaacgccttgagttgaagcgtttgtgtaagttaaaaggatggaggagaggggaagggttaggagatgatcaccagccttttaatgaaagcagcagcaatacacaagtccaattacaattatgtcttcctcaattgaagtcattgagaatagaaagatgcccattgctgacatttatgccgctgtgtcccaagacagaaaaactgcatttagttgtatttaatgaacgactccggatagtgcatgctaagagagatgagaatttctatgctccattacattcatcatcatctgatcctgaaaacccgaggaacactattcccattcccatgtttagagaggtatacataaacaatgtggcgtggctaaattcgctgcctatggaggcttttaggtgtctcactcatatgacaataaaaaacgacgaggtagagagtttgggagaagttggagaggtgtttcggagctgctcatcttctttgcgatccttgaatatcacaggttgctccaacttaagaagtgtttctggagggctggagcatctcactgctttggagatgttagaaatatacgacacccataagctgagtctatcagaagacccagaaggtgttgtgccatggaaatcccttcatcactccctcagctacttgcaactgatgaatctcccacagctggtcaacctgcctgattcgatgcagttcttggctgccctccgaactctttcaatagtgcattgcactaaactgcaatcagtgccagattggatgcccagactcacttctctcaggaagcttatggtttcattctgttccgcacatctggagagaagatgccaaaatccaactggggtggactggcctaacattcaacacatcccctccattgatgtcacctctagccttcctaagtttttagtgttgccgtatgaatag

SEQ ID NO: 2 - protein, 1163 aa, Beta vulgaris
MDVVGTALSAAQSLFAALQSSELKEILSIFGYKSRLDDLQRTVSTINAVFRDAETKQELTHEAQHWLEELKDAVFEADDLFDEFVTLAEQKQLVEAGGSLSKKMRQFFSDSNPLGIAYRMSRGVKKIKKKLDAIAYNHQFSFKIDLEPMKERRLETGSVVNAGDIIGREDDLEKIVGLLLDSNIQRDVSFLTIVGMGGLGKTALAQLVYNDPRVRTAFPLRCWNCVSDQDQKQLDVKEILGKILATATGKNHEGSTMDQVQTQLREQLCGKRYLLVLDDVWNENPNQLRDLVEFFMGGRSRNWIVVTTRSHETARIIRDGPLHKLQGLSEENSWRLFVRWTFGSVQAKFPNDFIMIARDIVDKCARNPLAIRVVGSLLCGQDKSKWLSFHEIDLGNIRKSHNDIMPILNLSYHHLEPPIKRCFSYCAVFPKDFLIGKQTLINLWMAQGYIVPLDKDQSIDDASEEYISILLRRCFFENVGAEKDGVIKIHDLMHDIAQNVMGKELCTTKNISGSLDKSVRHLSLARTSFARYSFNATHIRSYFCAGYWCQDAEINQFSVEALVPNCLYLRAMDLAWSKIKSLPDSIGGLLHLRYLDLSYNEDLEVLPNSIAKLYNLQTLQLKGCKRLEGLPKHLSRLVKLQTLDIHGCNNVTYMPKGMGKLTCLHTLSKFIVGGEGSCSSWKQCFDGLEDLKALNNLKGHLEIQIRWPKNTTDAVKEDVTREGLYLNHKEHLNHIVVDFRCEEGGGRMDDEEARRLMEELRPHPYLENLAVKAYYGVKMPGWATLLPNLTELFLSDCGELENLPCLGNLDHLKVLRLSHLAKLEYIEEDSSSANFRCRPGPESAGLSLYFPSLERLELKRLCKLKGWRRGEGLGDDHQPFNESSSNTQVQLQLCLPQLKSLRIERCPLLTFMPLCPKTEKLHLVVFNERLRIVHAKRDENFYAPLHSSSSDPENPRNTIPIPMFREVYINNVAWLNSLPMEAFRCLTHMTIKNDEVESLGEVGEVFRSCSSSLRSLNITGCSNLRSVSGGLEHLTALEMLEIYDTHKLSLSEDPEGVVPWKSLHHSLSYLQLMNLPQLVNLPDSMQFLAALRTLSIVHCTKLQSVPDWMPRLTSLRKLMVSFCSAHLERRCQNPTGVDWPNIQHIPSIDVTSSLPKFLVLPYE

SEQ ID NO: 3 - protein, 1177 aa, Beta vulgaris
MERVVYRWNTAETAGHLWPTNPKLILIPYSALQSSELKEILSIFGYKSRLDDLQRTVSTINAVFRDAETKQELTHEAQHWLEELKDAVFEADDLFDEFVTLAEQKQLVEAGGSLSKKMRQFFSDSNPLGIAYRMSRGVKKIKKKLDAIAYNHQFSFKIDLEPMKERRLETGSVVNAGDIIGREDDLEKIVGLLLDSNIQRDVSFLTIVGMGGLGKTALAQLVYNDPRVRTAFPLRCWNCVSDQDQKQLDVKEILGKILATATGKNHEGSTMDQVQTQLREQLCGKRYLLVLDDVWNENPNQLRDLVEFFMGGRSRNWIVVTTRSHETARIIRDGPLHKLQGLSEENSWRLFVRWTFGSVQAKFPNDFIMIARDIVDKCARNPLAIRVVGSLLCGQDKSKWLSFHEIDLGNIRKSHNDIMPILNLSYHHLEPPIKRCFSYCAVFPKDFLIGKQTLINLWMAQGYIVPLDKDQSIDDASEEYISILLRRCFFENVGAEKDGVIKIHDLMHDIAQNVMGKELCTTKNISGSLDKSVRHLSLARTSFARYSFNATHIRSYFCAGYWCQDAEINQFSVEALVPNCLYLRAMDLAWSKIKSLPDSIGGLLHLRYLDLSYNEDLEVLPNSIAKLYNLQTLQLKGCKRLEGLPKHLSRLVKLQTLDIHGCNNVTYMPKGMGKLTCLHTLSKFIVGGEGSCSSWKQCFDGLEDLKALNNLKGHLEIQIRWPKNTTDAVKEDVTREGLYLNHKEHLNHIVVDFRCEEGGGRMDDEEARRLMEELRPHPYLENLAVKAYYGVKMPGWATLLPNLTELFLSDCGELENLPCLGNLDHLKVLRLSHLAKLEYIEEDSSSANFRCRPGPESAGLSLYFPSLERLELKRLCKLKGWRRGEGLGDDHQPFNESSSNTQVQLQLCLPQLKSLRIERCPLLTFMPLCPKTEKLHLVVFNERLRIVHAKRDENFYAPLHSSSSDPENPRNTIPIPMFREVYINNVAWLNSLPMEAFRCLTHMTIKNDEVESLGEVGEVFRSCSSSLRSLNITGCSNLRSVSGGLEHLTALEMLEIYDTHKLSLSEDPEGVVPWKSLHHSLSYLQLMNLPQLVNLPDSMQFLAALRTLSIVHCTKLQSVPDWMPRLTSLRKLMVSFCSAHLERRCQNPTGVDWPNIQHIPSIDVTSSLPKFLVLPYE

SEQ ID NO: 4 - DNA, 987 bp, Beta vulgaris
ttcctctttagatttccatagatttgaacaaattggggtgattttcatagattattcataattctctctccataattcttctctctctttctccatacatttttcattcgcaatactcaggaactgagtattgggaattgtccccagttgtcaggttgatgtgcagtaactttaagagaagactttcctctcatgcaacatgtccctgatctgttgcttgatggtcgtcatctcactattctctaataagctcgatttgtatgaaacagatgatactatattccgtttcgtgcaatgtgcacgaaacggaatatagtattttgtgcaaggtgcacgaaacggattcgattgtttcgtgcacattgcacgaaacggaatcaactgtttcatgtagtctacacgaaacggaatcaattgtttcgtgtagtctacacgaaacagactaatcatgcattacgaatcataattacgaaaaaaaattaacaacttgaatcacaatgacgaaaaaaaattcagaaattatatcagattgaaattcgattgggtcaaaattatggtccattaaatatcaaattaaaatttgtagatcttcaatgaagttttttatatctaaccgttagagaggaggagagaatatttttagagagagaaagggttttttagaaagaatgtgataataagggttttttgggttttttttaggctgcgttagtaaagtgaggctgcatttagcaaccttttttttttggtaaatttcatttcctcgatgaacaaggaaacgaaacggcgagatggcggcgttggtggaatttcccggcgaaacgcagcttcctttcgattcatagttgccataaatttgcattttacccagatttcaaataatttttactaattcgctcaaattgctcatgaaattgtttatttccgcaaattttttgattaacccctccagaatttgattcgcaaatatggcgaagctattgagta

SEQ ID NO: 5 - DNA, 12364 bp, Beta vulgaris
ttctgttccgcacatctggagagaagatgccaaaatccaactggggtggactggcctaacattcaacacatcccctccattgatgtcacctctagccttcctaagtttttagtgttgccgtatgaataggtatatacttctttggttttggttcgtgcttccatttagctcaaattggaaatgagcgtatggcgtcagatggtgaccaatctgcagttattgcgctacgtgtatgttctggtttatattgatggcaatgttcaatagttcattataatcccaatcaaatttctttgtccattgtttataatcccaaatccaatttctttggaagattgtgctgaggagagcttgatgaaggaacttgtttaaggttttttctcttatagattatctttctaccattgtttataatcccaactgcatcttggtctgagaaggaattcaatattttttctagttttacttgaggttaaggctgtttataatcacaggctttgccaatagtataatttttataaagtactactgtacagattatgtgaatcttcaaaggtttgagagaatcgtcctaaattcatgtaaacttggagttaaggagcaggaaatggagttacttcaagtgttaatgcaatcagctcaaaaaattactaatacagaacttattcgtgtcacaactcagaagcctttataaattataaaagtagtaaagatttcgtttcgaaagtattattcatattagagtacaatgaataatttgctttggcaaagccatctgaaggtccttaagaaatgtttagtgcaggtgatttaacttgctgtgattatgtcaccaggagaacttgcttatcaaagaattcagtagcaagttggtcgatactcgacagaacatccttatcaaacatgttagtgcagaggtcagagcatgataccctttcattagtattatattttacattattaagaaatatatttacatctgaaattatatatgctgatacaataatcttatgcattttgagttatacattaaacacggtgaaaaacattatttcgagcatctgcatttgtgcttgtggttgtgtaatggtaaattggcaattgcttgacctttgtttaaggctgggtaagctttcaaaaagttgaattgtttagcagtagatcagtaactatccaaacaaagaccaagctatacgccaactgtttcttcacgttcactgtacaagtgttaaagtatcttcaatgggaataccgaaatctaaagtcaattatccaattaatagtagtcaaaagtcaaacatctctgtatgaatatgtagattgaagagtttctgtatgcattcaattcaatgcaacaagttgtattcgttcacaccttattacttggtcaaaagttgactaattttacacaaggaactttagcatcaatcatcatcctactatctacgagttgaaagaaacttgtacaaaaacttgttttaaccctgatacagttcagttaagcctgtttgttgatcagtctgcaatttgaatcactcgtccactcgcatgacttagtgtgcgatcttgtgtctagttttctcgagaccccgcctcctgaccgtgcccagcccaccccaaccattcccagctctactagctagtatcagcatacatgggaagagccaggactgtaagcatgtcgtttaccgagtcacagctgctgtcagcagcaggagatggagatgaggaattcctaatacaagctcttgctactcaacctattgattacttcctaacgcggagcaaaaacaaaaatggtgaagaacattgcaatattatccacattgcagtgttaaatgaacaagcaaagttcctcaatcgagcattgagtatattacccatctcaactctgcatctccttctctgtcagcaagatttttcctactttagctacaaccctcttcactgtgcatctttacgaggtaactttgctattgtcaagctcctcgtcgagttttacgaatcatcatcatcttcttcttcgtcattggttgatccaagctgtaagccatggttagccaaggatgtgaacgggaagacgcctttacaggtggctttggataggggtagaggtgaatgtgcattaaaaataatgggattagatgaagaattgctttgtaatatggttgataataaaggtaacagcccgctatttcaagctgtacaaagaggtagtgaacaaattgctatgaagatcttggcatcagggcattcttatagtactggtggcgagtatgagttgactccccttcatgttctaccaaattgctcaggtgtgtagtattgatttgtttttcaatttgttaaaatttcttacgctttctgtcccttaatttttctcacatgtgggtttgacacagacatttagtgttaagagcaacttcaatggtcagctatgcactcttctaacttagctttccacctcaactacattcaagtaacattagtttcaggctacaacgtccttttgggtgcatttcttcacttgaacttatatcaaaaccgagcttattactcttgattggacctaatcaaccatgatacgtgttttcgggaagttaacagtttcctaatttagttttcttctgtacaatttcaagataactaataaagtattagcaatcttaactataaaaaaagaagaaaacactagcctaatatcatctgatctgcagaggaagtttgcgaacttctacttgacaagcatccagaaatgataaaagcagtcgacaaaaatggacttacaatcctacacaaatgggcaatgatgggtaaactatggccatttcaatttcttttaaagcaagaaaaaagttctaggttgaggaaggacttcatcaaccttttatgtgcaactgagaagtcgacaggcaacaatcctttacacacagcagcttattaccacaatgaagaaactgcgcaggttgtgcagcttcttgtagaagcttatatagatgctaaggaacaaggagtggagcttcagccgagcccttggacatgtgagaatatagaaggagatacacctttgatggtatccttaatcaacaaacatgaaaaattggcactgtatttcatgtctgtggatatggagaattcagttgtatatgcaaccaagagtgtactatattgtgctgtactgcgtggatgtgatgaagttgcagaagaaacagtggcttcagttgatcctgcctgcttcagcttcatgcagcttaaagacgatggtgggcgaaatgtcttgcatgttgcatcaaattgcacaggtgaggtgagagtaccttattgcttgtatatctttcttcttatttgaaaaatcttggaggaactaagcacaagcaaggccaaggcttcgtcgtgctgtggtgggctcaaagaaggcctatgcacagcctggcccacatgggtgcaggcggcctctttaagaaattgaggaggccgaaacacggctggctttttgggcttgtgctcattttcaaaattgatgcccattacagcccacggagcactgctgtgatcttgtgtcgtgagtcatgacaggccagtaacgggcttgtgctgggcaagtaatatggcataactatccttatcattatttataaccggaacatctcatatatgcaaacctttaattctgactttgatcagtttattatagaacatggaaatcgaacatatctcagcagcatattcaagctattgtaaacttctttaaataattaaggtggtagacgtatatgccttgtattatttctggtcaaaatgagtatcagggaaatctaataaaacaatttaatctttacctatatagcaagaaaacagttgggattttgaaaacgggaaaatcttgagtcccatccatttatttgcttcattaccacggaactggggaaatttcacatacttgaagtttcggtgcttcatagattctaacattgaagtgtttatacagagagaacaggcaccttgttggtggaaaagctagcttggttgatcaacgagccagatgatgatggaaagagaccccttgatatagcttcagaagttggtaacgcatggcttataaaattactgctgacaaaagacccttcctcaaacacaagtgcgccatttgcttggattgaagcatgtaaaaaaggctacttatcagcaatacatgctttcatagaccattcccctgattttagaacattttgtctccaaagaaaagactctcctttacatcacatacaactgagaagttacaaagaataccaagaatttcttgctattccgttgattcaagagatgaaaaatatgctcgatttcagtggttcaacgcccttgcatcgagcattagaacgtaaggatatcctccttgctgaagcactgctctctggcgatggggttcatagaagcatcaaagataaaaatggtaaaactgctaccgacctgctagtaaagctgtgcgaccaagagtatgaatgggtatgtgtctccagtctccacctaattcttccaatctagaaaactatgattgcattaggaaatacttctatgtcagttgtcactatcatcccttgcttgctataagtctacattgtcttggcaaaaacataaaatgagcataaatataaaggttaattttttctagggaaattgtactgcgtataccctaaactagaatttgccaaataaccttagagattcaaaatatatccataactattaactttggctaatttgtaatggttctctcttatacaatttattgattcaaacctatttctgctgattaaacttgatcattggtaatattgaagaaaaattctcatggccttgcaagacagtgaagtttccatgaatctcggaaaaatgacagccacaggataaaataagactgctttagacagcatagtagctcttatgttttactatatacaagaatatgtaaaagccttgatctatgaaatgaattgttctatatatattattatggtgatatgcaagctccttctttgaattcaatttcaaacaaaatgcaggatactatgtgcaaacgtacacaaattagtccgtggctaacgacaaactatatcggaacttcccttgctaataaggcctttagatacacaggcagtacaagacttggtacaacaccatcagcaggagaaatgcgtagcacactttcagtcgtagcagcccttctagcaacccttacatttgcagctgggtttacacttcctggaggccttaacgaagatactggcgaagccatcttagcaaagaaggtttcatttctagtgtttatactagcagacacatacgcgatgtgttgctccatgttggtgctgttctgcctcatatggtctatggttagcgacagagataagtcacttctactgattgatcgaagtgttgtgatactcgtccaatcactttatggaacgttaatagcatttatggctggagtttacactgctatatcacacaagtctttgtgggcagctattatagtcattgttatgtgctctttcgttgcgatttcagctaacagagctattctggataaagtgcttgataagttgatcccttcggctgatagtaagagaagaaattaaacccagacactggatggatgtctggatgatgtaggctctcctataatctttcactatcttatgattttggatattactgtctgcaaatgttaaactcacacattgctattatagttctttgttatgcaagtatggattcaactctggactttggtcagtctggtaactagttgcagcccatgaccccaacttttagttattcttatactacctctgttttgtttataatacattggtacaaatcttattcatgttactagatgaacatgctaatgactagttttataatcggcttgttagatggagctctgagtacacatttgaaaaatatatctaattaaaaatattaaaccgactttaaacttgtacgatacatgagattataggaaataaagaatataagttttctaattattatacggttttaggaaaatttagcaattagtttagttattatattaatttgatacttagattttcaattagattatactagagtatataaaatttcctaattatatgtattcggttttcaatcagaaaataatgatttagttttattataaaattaaattactttttttagacggtgcttttctctccaaagtttcctcctttattcacacatgctaaacatggaagaatatatgtagcattattgttttcacacatcattttctaaaggttgtatgattcttattccaaagcaaattaccttcgataatgttgttactcgatatctaataaaaaacttttccatagatgatatcaagaccttaatgattttaataattatccaaataatcgccagagcaactagtactttttaaacaataatatattttttttgacaatggggtaaacaataatatttcttacataaacattttcatattcttagggggaaaaaccattaagaaaaatgcatgtatctattggatctctatacaagtttattttgatagttcgagccctaaattttgtcagcaagtcatatgtaagatttgtgtataaactataaagtgaactattgtttatttattagctatgaattaggtttcacaaaatattatataaagttgaatgatgattaacggaaactatactgatattatcatttgagattttctcttcatgtaaaagaccatttatcttatcccttatctctactagtctactttaagttcttgtgttatgtttaatttttgtcatgtatttacctaaatgctagttttacattcacaactccttttcttcactagagctatttaacatttcaaaatacgctataattttatattagcaaatataaacgtaatgatcgggattccttatattttttcacaaattattagaataggcggtctaatttttacataaattagatgaacttagaagtgaatttttcaaacaaacccattccatttcactctaacccaacactatcttagtcatcccttatcttttgcttcctttgttttcttgattctcgaactacaacagacaattttaagaaataactcggtatttttatcgaacggattaaactagtcactaaatggataaacaagtcactgaatgggttagtgaatgtcattcacgaaatagattaaattggtcacgaaatagagtcactatatttaaaaaggtggcatgttctctgctgaatattagacttgcaccgtgcctaattttaaaagtaggcgatatcttacaagacaactgtcatttttccacttccctaataatgagtaatcatgttcatgtatcatactccttgaacatgacatatatatttttctagaatgaaaaatcacctaacacaaaaaggggaaccaattagaaagagagaaagaaaagtaacacaaacaacaatcaaaacatgaaaacaactagcaaaatttattaagtactaattaatacatctagttacctaaaatgcactctaattactttaaaaagttcaaactccaacaatagtgcaaattagcataaacacttgttacagcaagttgtgcaaactcagacacacagaccacagaaggcggagtccccacaccagaggggcaactctaatttctccaacgtctcctttttctttctcttcttctcctttcatcttctttgctttctccctccagaatctttctctctcttccatttccaggtttctctctcctcttctctgcttcttattttttgaaagatgcaaacttttactgaaatttatgttttgaatagtgttacttattgttatgctttaaattctgagttgggtcactttcatttttgtttgaatttaatgggtttttgctgaattatgctctttttactccagtgaacggtttttcagtttctgggtgttaactgtatttagttaattaagattggtttgaattcaaaaaaaacttagggtttactattttccatgcttaatctttattttttaatgtctgaatatgtaaaaatgtaaaaattctatgttgaaaaactgagtaaaatagtatcaaatcaaagttttgaagctttgaattactgatatgttgtagtttggtacttggtttgatctgtgagattattcataagatgctatctttatttcctgttttctttttagtgcaaatattctgaataaaatatgcattagtttacttttatatagaatataagtatttgggattctaagttatgggacactcaattttatatgcagatccagctgttccagactagactaacttggtagcttgagcttcacttgttgtgcttggatctgttaagcttggaagttttgctgatttagcgccatatgttctagatgtattgtattagtcaagtaaagttttgatatcgaaatttggacctttagtggcataagagtggtttattcttcatttagaattttgaccttgagcttagttttggaattgagtggttgagaaacttcaaacactttggcttttcagtttattatacccgggtttttattgaggaaggtagtgagaaagctccaggaaaatttgactcttgtgtctacagaaaagtcacttagtcttctcctataattttgctgtaatcctggttctggacctctaggctctggaatggcagttggcaaaaacagcagtaacgctggatcattaactcggccatgtcattgtttcaaggtggcaaacttgaaggaaactattttggatgctagcgagacatccgagttaaaagatcgttatgttttgggagatcaactaggttgggggcagtttggtgtgatccgggcatgtgctgataagtttactggagaactactggcgtgcaagtccattgccaaagatagacttgtaacacaagatgatgttcgaagtgtgaagctcgaaatcgagattatgagcaagttgtccggtcatcctcatgttgtcgatctcaaagctgtttatgaggaagaagattatgtccacttggtgatggagctttgtgccggtggggagttgttccaccgattagagaaacaaggaaggtattgcgagtctcaagccaaagtcatcttcaggcatctaatgcaagtagtcttgtattgtcatgataatggtgttgttcatagagatttgaagcctgaaaatgttcttttggcaaccaagtcttcttcttcgccaattaaattagccgattttggtcttgctacatatatcaaaccaggtagaacactcttcttcatctagtttgtgattttagctgtgttactcggtctctttcaattcacctcaatagctgtccatgttgaattttggataatttgatcaagtcagtctggcccctaaacatgttcctgcgcccaacactaacagtgtcttaagcctttggttactggtcaagcaggggagagtttgcatgggacagtggggagtcctttctatatagctcctgaagttctgtcaggaggttacacccaggctgctgatgtatggagtgctggcgtaattctctacattctcttgagttctatgccaccattttgggggaagacaaagtcaaggatatttgatgcagttcgagcagctgatctgcgcttcccttctgaactttgggatcggatatcagaacctgccaaggagctgatcaggaaaatgctttgtgtagatcctttgaagcgcttgacagctgagcaagttttaggtatatttttaatttttgcctcctttgctgaattcagatgacagttatatgacacagtatacatttgtagaacccaagtgtctgaatagccaatcaccaatgtctgacaagttttttttggctttcgattacaaaatcatttattacatatttgcattaactgtgttatttttgacacattacatgaaatcttcattgcttatttgtgattctttgtgaattgctgtacattggaagctgctcccttttaacatttgagatgtccgtaagtggtgagtgtaactcatctgtccccacggagacaaagcttttggatgattttaggacaaatgcatttaacgttctcagcttatctgacaatgttatccatggtgtccgtggacacatgtaccaacactaaacatctagtatttcttgttggttctttagttttgctggatatacttaagggctaaggctttatttttgttcctgcagctcactcatggatggaagaggttactgtagctacggaagaatcacatgaacatgatttggcctgctctgaacatttaaaaacccgagatagctcattttcagcgtcatgtatatccagggatcacgatataagctttggcactggatctgcggtaaattgtgaacctcaatctccaacatttacgtgcagatcttcattctcggcatttatggcggaaccatccacccctacccttatatctgctggattttctttccgtagcagcggtgatttcactgctcttgagtttgtttctccaattccttccttgcctagcttcacatttttcagccctaggtcagtagatgagcatggaaaccaaaataaggttttttcaagcaacagggagaacactgacgaaattcatacaggtaactcacttttctatttgtaataatttgttattgtcactgattctctaatgtcatttttgcatctctaggtcttgtaacattttaaacgtcatataaacatccatgacattttatgtattttgctcaactttcaagtatttttgtatgacttttaaactttcaagttttatctgcgtataacttttcatagcctaaccgtttctctgttgtataagtatatgcgaaaaatcattcatcacatgaattgtttgaatctaatgttggattgtgcagcctaaccaactcgagtttcttaaaaaaaattgttctgtaattcaattatgtcctccatatcttatctttctttacttttaaagcactattgagaaacagaagaaaaccccagtgtgacgactgtcagatgtggtttgattgagattagactattttatcagtgttgtgttattgagattccagtgctgttaatatcattagttccatcgtaagcttttaaagttatcaattcataaaactagatctaatgcccatcgtatttttagaaggggccgacttggagaagcgatttgaatcacctcattcatcgctgtgctcaggaattgatgctagggacctgaaagagaagtcagcagactctaagaggagtggaggaacaggggtgaggatttttgggatccataacaagagaaataggacgattgggcttggcgaattcaaccagcttgatattgtggtcactgaatctgtcatccgatgggcgtcatgcacccacttacctaccgcctcatcactcaggtcttctcttgtatgctgataatcatgggccgaccacaatgtatcaaattaacatcataaatcatgatataaagttgggcaacacgcaaacgtgtgaattctactgctctgctacaagattgaagatataatgggtttgagtcgcgtgtactgttggtgatgatcatcccatattagagagctaaatgttagtaactacattgtaatggatctgcagaataagcagattcttcttcaaaaggtgtaaagcatggattttgaaagcaatggttttctcaacctttttgatcatgatttagtagatatatatagggggctttttgttcttattagatgtgattgttaagccttcttcatgaacaaacataagcactggtgacttgtgggatggtacatagaaagagttccgtttcatcgattttgattttgtccagatcctccttttctttcgaaaaaagggaaggagagtatccgaaagattacccattttgtattttcggttgtctttaaaagattgatccattacctttcggacaatttgattcctataatactcctatttctctacttcatttcctgccatatactactatactaaagacaaaattacttaatacgaacttaaaattaagaggagaaacaaggtaaaatttggtgaggatgatggaggaatcatatgaaagcttacgcacattatatatttgggagtatgatgtacactagttaatgaagatcagacacttttctatatcttttgattcgtatgttctttaataaatgaagatggtatatttaaaatttcgtgtgtatttgaaaatatcatgcacattagacatccaagtctaagattaattcacaactatctattttttttt

SEQ ID NO: 6 - DNA, 4659 bp, Beta vulgaris
  misc_feature (461)..(485): n is a, c, g, or t
  misc_feature (621)..(696): n is a, c, g, or t
  misc_feature (704)..(707): n is a, c, g, or t
  misc_feature (1115)..(1123): n is a, c, g, or t
  misc_feature (1169)..(1170): n is a, c, g, or t
  misc_feature (1879)..(1880): n is a, c, g, or t
  misc_feature (2194)..(2194): n is a, c, g, or t
caaatcttctggcatcaatggcggtgttgccgttcatcawtttaacatcaatggaggtaagagtcatgttttttcaacaatataaaacttatatgatttttctgtttttccccgtatcttgtttgagattgtgattattaagagagtcaagtctcacaatattcgaaagtctacgtaatccacctcaaattgacgaagaaaacaagcaggaaaggattaagtaagttcgtggaaccaytagaattaattttcaaatatagctctacctaatatatggcctacttttaattttaaataagaagaaggtaatgtgattagaaacaaattggtcttaaattattcattaagcttaataatgcataaactttatcaagtgctatcttcttttcagggccgtcttgaagattttkggkcccrgttctattatgaaaattgrgcccctaaatttatasaaaataaannnnnnnnnnnnnnnnnnnnnnnnngatggaaggttagagyyctaaagatagaaagttgaaaatctaaatataaatcattgacaaatttattaagggtgagaaacaagggtgttttcttcaaatatgaagcaaaattttcaaaataatatawtttkggscnnnnnnnnnnnnnnnnnnnnnnnnnnnnnnnnnnnnnnnnnnnnnnnnnnnnnnnnnnnnnnnnnnnnnnnnnnnncttctttnnnntgatacaatttttsagcgacatgattgtcgattgatgcttatattattgtatactcgatccatattgtttaagatgaattgtttgtctttgatggtctccaatgcatattttgtatwmttaggaattytaattatgtactattagtasayatygagaygaatacaraatygccataatgaagtatgattattttarttatatactttctccgttccaaatatataartgtaacacttgtgtactttatgcgtactaatgcataayaacgtgcactctccygtgtttaattatatactttttgagagaagtgwtacattggggaccatgggactgtgtataatttgaccgcaaaatygaagtgtygcatttgattgaaaayggagarrgtagtatatagrtggaacacnnnnnnnnntgctgrtcatctttggccaacaaaccmaaaattgatattaatccynntwwtymrgkwyttttcatctttttgacacaaaatggatgttgtaggcwctgcgctatctgctgcccaatctctgtttgcagccctgcaaagttctgagctcaaagagatcctctcgatctttggctacaaatcccaacttgatgacctccaacgcaytgtmtctaccatcaaygctgtattccgtgatgctgagaccaaacaggagctcactcatgaagcacarcattggctcgaggaactcaaggatgctgtctttgaagcagatgatctgttcgacgagtttgtcactcttgccgagcagaagcaacttgtagaggctggtggcagtctttccaaaaagatgcgccaattcttttctgattccaacccccttggcatygcttatargatgtcacraggggttaagaagatcaagaagaagttggatgytatygcttacaatcatcaatttagctttaagattgatcttgagcctataaaagagagaaggctcgagactggttctgtcgtgaacgcaggtgatatcattggaagagaggatgacttggagaagatcgtaggtttgttkcttgattctaacatccagcgtgatgtgtctttccttackatwgtgggaatgggagggttgggtaaaactgctcttgcccaactcgtgtacaatgatccaagggtcagaactgcttttccattgagatgttggaattgtsnntctgatcaagatcaaaakmaactagatgtgaaagaaattttgggtaagattctgtctacagctactggtaagaatcayragggttcaaccatggatcakgtgcaaaccyaactacrrgaacaactatgtggcaagagatacttgcttgttttggatgatgtatggaatgagaatcctaatcaattgcgtrwyytkgkwraattcttcatgggaggtcaaaggggaaattggattstggtaactacgcgttcgcaygagacarcgagaattataagagatggtccattgcacaagctscaaggtttgtctgarrnaaaactyttggcgtttatytgtaaggtggaccttcggatcagtgcaaccaaaattccctaatgactttgtcatgattgcacgagatatagtygacaaatgtgctcgaaaccctytggctataagagtggtaggaagtcttttgtgtggtcaagacaagagtaagtggctttcatttcatgagatmtgtttagccaacattagaaagagycataatgatatcatgcyaatactgaacctaagttaccatcatcttgaacctccaatcakgagatgctttagttattgtgcartgtttccaaaggatttccttatagggaagaagacgttgataaacctttggatggcacaaggttatattgttccattagacaaagatcaaagcatagatgaygctagtgaggaatacatatcaattttgytgcagagatgttttttcgaaaacatcggaacagaaaaagatkatgttattaagatacatgatctcatgcatgatattgctcaaaatgtcatggggaaggagctttgtacgacaaaaaacattagtggcagcttggataaaaatgttcgccatctatctcttgccagaactagttttgcaagatactctttyaatgcaactcatattcgctccyatttctrtgctggctactggtgtcaggawkctgagataamccagttytcagttgaggcattagtaccaaaytgtttgtgcctaagggcattgkacctsgcttggtcgaagataaaaagtktaccagactcrattggtggattgttgcatttgaggtacttagatctttcrtataasgaagatytggaagtacttccgaactcaattgcyaaactatataatctrcaaaccttacaattgaagggttgcaagagattggaagggttaycaaaacatttgagcaggctggttaagcttcaaactttrgatatatatggttgcaayaatgtaacttatatgcccaaaggcatgggtaagatgacttgccttcacactctcagtaagtttatagtgggtggagaagggarttgttcaagttggaagmaayggtttgatgggcwggaagatctaaaggctctcaacaacctaaagggtcatctggraatccaaatcaggtggcccgaaaatactacagatgctgtcaaggaagatgttaagagggaaggattatacytgaatcataaggaacatctcaatcacattgtggttgatttcagatgtgaggagggtggtggaagaatggatgatgaggaagcaagaagattgatggaagagytgcggccacatccttatcttgaaaatttggctgtgaaagcataytatggtgygaaaaygcctgrttgggyaacccttctyccaaatcttacagagctttwtctttytgattgtggggaayyggagwrccttccatgcmtgggaaacttggwtydtctraamgtyctccgrctttcgcatttggcraaattggagtayattgragaagatagcwcatcagctmwtttcagktktaggcctggaccrgaaagtgcaggactatcattatacttcccctcccttgaackccttgagttgaagcrtttgyryaagttaaaaggatggaggagargggaagggttaggagatgatcaccagccttttaatgaaagcagcagcaataagtcattgagaatagaaagatgcccattgctgacatttatgccgctgtgtcccaagacagaaaaacdgcatttagttgtatttaatgaaygactccggatagtgcatactaaaggagatgagaatttctatgctccattacattcatcatcatctgatcctgaaaacccgaggagcactattcccattcccatgttaagagaggtatacataaacaatgtggcatggctaaattcgctgcctatggaggcttttaggtgtctcactcatatgacaataaaaaacgacaaggtagagagtttgggagaagttggggaggtgtttcggagctrctcatcttctttgcgatccttgaatatcacaggttgctccaacttaagaagtgtttctggagggctggagcatctcactrctttggagatkttagaaatatacgacacccataagctgagtctwtcagaagacccagaaggtgttgtgccatggaaatcccttcatcactccctcagctacttgmaattgatgaatctcccwcagctggtcaacctgcctgattcgatgcagttcttggyctccctccaaaccctttcaatggtgcattgcagtaaactggaatcagtgccagattggatgcccmgactcacttcyctcaggaagcttatggtttcattctgttccgcacatctggagagaagatgycaaaatccaactggggtggactggcctaacattcaacacatcccctscattgatgtcacctctagccgtcctaagtttttagtgttgccgtatgaatag

SEQ ID NO: 7 - DNA, 434 bp, Beta vulgaris
gaactcaaggatgctgtctttgaagcagatgatctgttcgacgagtttgtcactcttgccgagcagaagcaacttgtagaggctggtggcagtctttccaaaaagatgcgccaattcttttctgattccaacccccttggcattgcttataggatgtcacgaggggttaagaagatcaagaagaagttggatgctatcgcttacaatcatcaatttagctttaagattgatcttgagcctatgaaagagagaaggctagagactggttctgtcgtgaacgcaggtgatatcattggaagagaggacgacttggagaagattgtaggtttgttgcttgattctaacatccaacgtgatgtgtctttccttactattgtgggaatgggagggttgggtaaaactgctcttgcccaactcgtgtacaatgatccaag